European Patent Application EP 4 814 132 A1, published September 30, 2026. Title: 반려동물의 PIK3CA 유전자 돌연변이성 종양 검출용 조성물 및 이를 이용한 반려동물의 PIK3CA 유전자 돌연변이성 종양 진단방법. Applicant: 홍재우. The sequence listing filed with the application follows.

SEQUENCE LISTING (8 sequences)

SEQ ID NO: 1 - DNA, 22 bp, synthetic construct
  source 1..22: mol_type = other DNA
gatcctctctctgaaatcactg

SEQ ID NO: 2 - DNA, 22 bp, synthetic construct
  source 1..22: mol_type = other DNA
gatcctctctctgaaatcacta

SEQ ID NO: 3 - DNA, 22 bp, synthetic construct
  source 1..22: mol_type = other DNA
catacattcgaaagaccctagc

SEQ ID NO: 4 - DNA, 21 bp, synthetic construct
  source 1..21: mol_type = other DNA
aggttagtaccaatgcagcgt

SEQ ID NO: 5 - DNA, 21 bp, synthetic construct
  source 1..21: mol_type = other DNA
tgttgtccagccaccatgatg

SEQ ID NO: 6 - DNA, 21 bp, synthetic construct
  source 1..21: mol_type = other DNA
ttgttgtccagccaccatgag

SEQ ID NO: 7 - DNA, 21 bp, synthetic construct
  source 1..21: mol_type = other DNA
ttgttgtccagccaccatgaa

SEQ ID NO: 8 - DNA, 21 bp, synthetic construct
  source 1..21: mol_type = other DNA
tgttgtccagccaccatgata